European Patent Specification EP 3 503 927 B1, published February 19, 2025. Title: Topical Formulations based on Ionic Species for Skin Treatment. Applicant: University of California, Santa Barbara Zakrewsky, Michael Mitragotri, Samir. The sequence listing filed with the application follows.

SEQUENCE LISTING (12 sequences)

SEQ ID NO: 1 - RNA, 21 nt, Artificial Sequence
  FAM-GAPDH siRNA, shown 5' to 3'
  misc_feature (1)..(1): 5' FAM modification
gacguaaacggccacaaguuc

SEQ ID NO: 2 - RNA, 21 nt, Artificial Sequence
  FAM-GAPDH siRNA, shown 5' to 3'
  misc_feature (1)..(1): 5' FAM modification
gugugaaccacgagaaauauu

SEQ ID NO: 3 - RNA, 21 nt, Artificial Sequence
  FAM-Elastase siRNA, shown 5' to 3'
  misc_feature (1)..(1): 5' FAM modification
ucacuuacaggaucuauaauu

SEQ ID NO: 4 - RNA, 21 nt, Artificial Sequence
  FAM siRNA, shown 5' to 3'
  misc_feature (1)..(1): 5' FAM modification
uaaggcuaugaagagauacuu

SEQ ID NO: 5 - RNA, 23 nt, Artificial Sequence
  siRNA sequence for GAPDH, shown 5' to 3'
gacguaaacggccacaaguucuu

SEQ ID NO: 6 - RNA, 23 nt, Artificial Sequence
  siRNA sequence for GAPDH, shown 5' to 3'
gaacuuguggccguuuacgucuu

SEQ ID NO: 7 - RNA, 23 nt, Artificial Sequence
  siRNA sequence for GAPDH - shown 5' to 3'
gugugaaccacgagaaauauuuu

SEQ ID NO: 8 - RNA, 23 nt, Artificial Sequence
  siRNA sequence for GAPDH, shown 5' to 3'
aauauuucucgugguucacacuu

SEQ ID NO: 9 - RNA, 21 nt, Artificial Sequence
  siRNA sequence for elastase, shown 5' to 3'
ucacuuacaggaucuagaauu

SEQ ID NO: 10 - RNA, 21 nt, Artificial Sequence
  siRNA sequence for elastase, shown 5' to 3'
uuauagauccuguaagugauu

SEQ ID NO: 11 - RNA, 21 nt, Artificial Sequence
  non-silencing siRNA control sequence, shown 5' to 3'
uaaggcuaugaagagauacuu

SEQ ID NO: 12 - RNA, 21 nt, Artificial Sequence
  non-silencing siRNA control sequence, shown 5' to 3'
guaucucuucauagccuuauu